European Patent Application EP 4 166 155 A1, published April 19, 2023. Title: Composition comprising pentapeptide as an active ingredient. Applicant: CAREGEN CO., LTD. The sequence listing filed with the application follows.

SEQUENCE LISTING (11 sequences)

SEQ ID NO: 1 - protein, 5 aa, Artificial Sequence
  Pentapeptide
KFLIK

SEQ ID NO: 2 - DNA, 20 bp, Artificial Sequence
  Forward primer for IL-1alpha
gaagtcaggcagaagtgctc

SEQ ID NO: 3 - DNA, 20 bp, Artificial Sequence
  Reverse primer for IL-1alpha
gtgcacccgactttgttctt

SEQ ID NO: 4 - DNA, 20 bp, Artificial Sequence
  Forward primer for TNF-alpha
cgtcagccgatttgctatct

SEQ ID NO: 5 - DNA, 20 bp, Artificial Sequence
  Reverse primer for TNF-alpha
cggactccgcaaagtctaag

SEQ ID NO: 6 - DNA, 20 bp, Artificial Sequence
  Forward primer for IL-1beta
caaggagaaccaagcaacga

SEQ ID NO: 7 - DNA, 20 bp, Artificial Sequence
  Reverse primer for IL-1beta
ttggccgaggactaaggagt

SEQ ID NO: 8 - DNA, 20 bp, Artificial Sequence
  Forward primer for COX-2
tgagtggtagccagcaaagc

SEQ ID NO: 9 - DNA, 20 bp, Artificial Sequence
  Reverse primer for COX-2
ctgcagtccaggttcaatgg

SEQ ID NO: 10 - DNA, 20 bp, Artificial Sequence
  Forward primer for GAPDH
accacagtccatgccatcac

SEQ ID NO: 11 - DNA, 20 bp, Artificial Sequence
  Reverse primer for GAPDH
tccaccaccctgttgctgta